European Patent Specification EP 3 963 062 B1, published January 7, 2026. Title: Lipid-Encapsulated Dual-Cleaving Endonuclease for DNA and Gene Editing. Applicant: Specific Biologics Edgell, David R MacMurrough, Thomas R Stead, Brent R Israel, Odisho R. The sequence listing filed with the application follows.

SEQUENCE LISTING (20 sequences)

SEQ ID NO: 1 - DNA, 4440 bp, Homo sapiens
atgcagaggtcgcctctggaaaaggccagcgttgtctccaaactttttttcagctggaccagaccaattttgaggaaaggatacagacagcgcctggaattgtcagacatataccaaatcccttctgttgattctgctgacaatctatctgaaaaattggaaagagaatgggatagagagctggcttcaaagaaaaatcctaaactcattaatgcccttcggcgatgttttttctggagatttatgttctatggaatctttttatatttaggggaagtcaccaaagcagtacagcctctcttactgggaagaatcatagcttcctatgacccggataacaaggaggaacgctctatcgcgatttatctaggcataggcttatgccttctctttattgtgaggacactgctcctacacccagccatttttggccttcatcacattggaatgcagatgagaatagctatgtttagtttgatttataagaagactttaaagctgtcaagccgtgttctagataaaataagtattggacaacttgttagtctcctttccaacaacctgaacaaatttgatgaaggacttgcattggcacatttcgtgtggatcgctcctttgcaagtggcactcctcatggggctaatctgggagttgttacaggcgtctgccttctgtggacttggtttcctgatagtccttgccctttttcaggctgggctagggagaatgatgatgaagtacagagatcagagagctgggaagatcagtgaaagacttgtgattacctcagaaatgattgaaaatatccaatctgttaaggcatactgctgggaagaagcaatggaaaaaatgattgaaaacttaagacaaacagaactgaaactgactcggaaggcagcctatgtgagatacttcaatagctcagccttcttcttctcagggttctttgtggtgtttttatctgtgcttccctatgcactaatcaaaggaatcatcctccggaaaatattcaccaccatctcattctgcattgttctgcgcatggcggtcactcggcaatttccctgggctgtacaaacatggtatgactctcttggagcaataaacaaaatacaggatttcttacaaaagcaagaatataagacattggaatataacttaacgactacagaagtagtgatggagaatgtaacagccttctgggaggagggatttggggaattatttgagaaagcaaaacaaaacaataacaatagaaaaacttctaatggtgatgacagcctcttcttcagtaatttctcacttcttggtactcctgtcctgaaagatattaatttcaagatagaaagaggacagttgttggcggttgctggatccactggagcaggcaagacttcacttctaatggtgattatgggagaactggagccttcagagggtaaaattaagcacagtggaagaatttcattctgttctcagttttcctggattatgcctggcaccattaaagaaaatatcattggtgtttcctatgatgaatatagatacagaagcgtcatcaaagcatgccaactagaagaggacatctccaagtttgcagagaaagacaatatagttcttggagaaggtggaatcacactgagtggaggtcaacgagcaagaatttctttagcaagagcagtatacaaagatgctgatttgtatttattagactctccttttggatacctagatgttttaacagaaaaagaaatatttgaaagctgtgtctgtaaactgatggctaacaaaactaggattttggtcacttctaaaatggaacatttaaagaaagctgacaaaatattaattttgcatgaaggtagcagctatttttatgggacattttcagaactccaaaatctacagccagactttagctcaaaactcatgggatgtgattctttcgaccaatttagtgcagaaagaagaaattcaatcctaactgagaccttacaccgtttctcattagaaggagatgctcctgtctcctggacagaaacaaaaaaacaatcttttaaacagactggagagtttggggaaaaaaggaagaattctattctcaatccaatcaactctatacgaaaattttccattgtgcaaaagactcccttacaaatgaatggcatcgaagaggattctgatgagcctttagagagaaggctgtccttagtaccagattctgagcagggagaggcgatactgcctcgcatcagcgtgatcagcactggccccacgcttcaggcacgaaggaggcagtctgtcctgaacctgatgacacactcagttaaccaaggtcagaacattcaccgaaagacaacagcatccacacgaaaagtgtcactggcccctcaggcaaacttgactgaactggatatatattcaagaaggttatctcaagaaactggcttggaaataagtgaagaaattaacgaagaagacttaaaggagtgcttttttgatgatatggagagcataccagcagtgactacatggaacacataccttcgatatattactgtccacaagagcttaatttttgtgctaatttggtgcttagtaatttttctggcagaggtggctgcttctttggttgtgctgtggctccttggaaacactcctcttcaagacaaagggaatagtactcatagtagaaataacagctatgcagtgattatcaccagcaccagttcgtattatgtgttttacatttacgtgggagtagccgacactttgcttgctatgggattcttcagaggtctaccactggtgcatactctaatcacagtgtcgaaaattttacaccacaaaatgttacattctgttcttcaagcacctatgtcaaccctcaacacgttgaaagcaggtgggattcttaatagattctccaaagatatagcaattttggatgaccttctgcctcttaccatatttgacttcatccagttgttattaattgtgattggagctatagcagttgtcgcagttttacaaccctacatctttgttgcaacagtgccagtgatagtggcttttattatgttgagagcatatttcctccaaacctcacagcaactcaaacaactggaatctgaaggcaggagtccaattttcactcatcttgttacaagcttaaaaggactatggacacttcgtgccttcggacggcagccttactttgaaactctgttccacaaagctctgaatttacatactgccaactggttcttgtacctgtcaacactgcgctggttccaaatgagaatagaaatgatttttgtcatcttcttcattgctgttaccttcatttccattttaacaacaggagaaggagaaggaagagttggtattatcctgactttagccatgaatatcatgagtacattgcagtgggctgtaaactccagcatagatgtggatagcttgatgcgatctgtgagccgagtctttaagttcattgacatgccaacagaaggtaaacctaccaagtcaaccaaaccatacaagaatggccaactctcgaaagttatgattattgagaattcacacgtgaagaaagatgacatctggccctcagggggccaaatgactgtcaaagatctcacagcaaaatacacagaaggtggaaatgccatattagagaacatttccttctcaataagtcctggccagagggtgggcctcttgggaagaactggatcagggaagagtactttgttatcagcttttttgagactactgaacactgaaggagaaatccagatcgatggtgtgtcttgggattcaataactttgcaacagtggaggaaagcctttggagtgataccacagaaagtatttattttttctggaacatttagaaaaaacttggatccctatgaacagtggagtgatcaagaaatatggaaagttgcagatgaggttgggctcagatctgtgatagaacagtttcctgggaagcttgactttgtccttgtggatgggggctgtgtcctaagccatggccacaagcagttgatgtgcttggctagatctgttctcagtaaggcgaagatcttgctgcttgatgaacccagtgctcatttggatccagtaacataccaaataattagaagaactctaaaacaagcatttgctgattgcacagtaattctctgtgaacacaggatagaagcaatgctggaatgccaacaatttttggtcatagaagagaacaaagtgcggcagtacgattccatccagaaactgctgaacgagaggagcctcttccggcaagccatcagcccctccgacagggtgaagctctttccccaccggaactcaagcaagtgcaagtctaagccccagattgctgctctgaaagaggagacagaagaagaggtgcaagatacaaggctttag

SEQ ID NO: 2 - DNA, 3261 bp, Homo sapiens
atgcgaccctccgggacggccggggcagcgctcctggcgctgctggctgcgctctgcccggcgagtcgggctctggaggaaaagaaagtttgccaaggcacgagtaacaagctcacgcagttgggcacttttgaagatcattttctcagcctccagaggatgttcaataactgtgaggtggtccttgggaatttggaaattacctatgtgcagaggaattatgatctttccttcttaaagaccatccaggaggtggctggttatgtcctcattgccctcaacacagtggagcgaattcctttggaaaacctgcagatcatcagaggaaatatgtactacgaaaattcctatgccttagcagtcttatctaactatgatgcaaataaaaccggactgaaggagctgcccatgagaaatttacagggacaaaagtgtgatccaagctgtcccaatgggagctgctggggtgcaggagaggagaactgccagaaactgaccaaaatcatctgtgcccagcagtgctccgggcgctgccgtggcaagtcccccagtgactgctgccacaaccagtgtgctgcaggctgcacaggcccccgggagagcgactgcctggtctgccgcaaattccgagacgaagccacgtgcaaggacacctgccccccactcatgctctacaaccccaccacgtaccagatggatgtgaaccccgagggcaaatacagctttggtgccacctgcgtgaagaagtgtccccgtaattatgtggtgacagatcacggctcgtgcgtccgagcctgtggggccgacagctatgagatggaggaagacggcgtccgcaagtgtaagaagtgcgaagggccttgccgcaaagtgtgtaacggaataggtattggtgaatttaaagactcactctccataaatgctacgaatattaaacacttcaaaaactgcacctccatcagtggcgatctccacatcctgccggtggcatttaggggtgactccttcacacatactcctcctctggatccacaggaactggatattctgaaaaccgtaaaggaaatcacagggtttttgctgattcaggcttggcctgaaaacaggacggacctccatgcctttgagaacctagaaatcatacgcggcaggaccaagcaacatggtcagttttctcttgcagtcgtcagcctgaacataacatccttgggattacgctccctcaaggagataagtgatggagatgtgataatttcaggaaacaaaaatttgtgctatgcaaatacaataaactggaaaaaactgtttgggacctccggtcagaaaaccaaaattataagcaacagaggtgaaaacagctgcaaggccacaggccaggtctgccatgccttgtgctcccccgagggctgctggggcccggagcccagggactgcgtctcttgccggaatgtcagccgaggcagggaatgcgtggacaagtgcaaccttctggagggtgagccaagggagtttgtggagaactctgagtgcatacagtgccacccagagtgcctgcctcaggccatgaacatcacctgcacaggacggggaccagacaactgtatccagtgtgcccactacattgacggcccccactgcgtcaagacctgcccggcaggagtcatgggagaaaacaacaccctggtctggaagtacgcagacgccggccatgtgtgccacctgtgccatccaaactgcacctacggatgcactgggccaggtcttgaaggctgtccaacgaatgggcctaagatcccgtccatcgccactgggatggtgggggccctcctcttgctgctggtggtggccctggggatcggcctcttcatgcgaaggcgccacatcgttcggaagcgcacgctgcggaggctgctgcaggagagggagcttgtggagcctcttacacccagtggagaagctcccaaccaagctctcttgaggatcttgaaggaaactgaattcaaaaagatcaaagtgctgggctccggtgcgttcggcacggtgtataagggactctggatcccagaaggtgagaaagttaaaattcccgtcgctatcaaaacatctccgaaagccaacaaggaaatcctcgatgaagcctacgtgatggccagcgtggacaacccccacgtgtgccgcctgctgggcatctgcctcacctccaccgtgcagctcatcacgcagctcatgcccttcggctgcctcctggactatgtccgggaacacaaagacaatattggctcccagtacctgctcaactggtgtgtgcagatcgcaaagggcatgaactacttggaggaccgtcgcttggtgcaccgcgacctggcagccaggaacgtactggtgaaaacaccgcagcatgtcaagatcacagattttgggctggccaaactgctgggtgcggaagagaaagaataccatgcagaaggaggcaaagtgcctatcaagtggatggcattggaatcaattttacacagaatctatacccaccagagtgatgtctggagctacggggtgaccgtttgggagttgatgacctttggatccaagccatatgacggaatccctgccagcgagatctcctccatcctggagaaaggagaacgcctccctcagccacccatatgtaccatcgatgtctacatgatcatggtcaagtgctggatgatagacgcagatagtcgcccaaagttccgtgagttgatcatcgaattctccaaaatggcccgagacccccagcgctaccttgtcattcagggggatgaaagaatgcatttgccaagtcctacagactccaacttctaccgtgccctgatggatgaagaagacatggacgacgtggtggatgccgacgagtacctcatcccacagcagggcttcttcagcagcccctccacgtcacggactcccctcctgagctctctgagtgcaaccagcaacaattccaccgtggcttgcattgatagaaatgggctgcaaagctgtcccatcaaggaagacagcttcttgcagcgatacagctcagaccccacaggcgccttgactgaggacagcatagacgacaccttcctcccagtgcctggtgagtggcttgtctggaaacagtcctgctcctcaacctcctcgacccactcagcagcagccagtctccagtgtccaagccaggtgctccctccagcatctccagagggggaaacagtggcagatttgcagacacagtga

SEQ ID NO: 3 - DNA, 3260 bp, Homo sapiens
atgcgaccctccgggacggccggggcagcgctcctggcgctgctggctgcgctctgcccggcgagtcgggctctggaggaaaagaaagtttgccaaggcacgagtaacaagctcacgcagttgggcacttttgaagatcattttctcagcctccagaggatgttcaataactgtgaggtggtccttgggaatttggaaattacctatgtgcagaggaattatgatctttccttcttaaagaccatccaggaggtggctggttatgtcctcattgccctcaacacagtggagcgaattcctttggaaaacctgcagatcatcagaggaaatatgtactacgaaaattcctatgccttagcagtcttatctaactatgatgcaaataaaaccggactgaaggagctgcccatgagaaatttacagggacaaaagtgtgatccaagctgtcccaatgggagctgctggggtgcaggagaggagaactgccagaaactgaccaaaatcatctgtgcccagcagtgctccgggcgctgccgtggcaagtcccccagtgactgctgccacaaccagtgtgctgcaggctgcacaggcccccgggagagcgactgcctggtctgccgcaaattccgagacgaagccacgtgcaaggacacctgccccccactcatgctctacaaccccaccacgtaccagatggatgtgaaccccgagggcaaatacagctttggtgccacctgcgtgaagaagtgtccccgtaattatgtggtgacagatcacggctcgtgcgtccgagcctgtggggccgacagctatgagatggaggaagacggcgtccgcaagtgtaagaagtgcgaagggccttgccgcaaagtgtgtaacggaataggtattggtgaatttaaagactcactctccataaatgctacgaatattaaacacttcaaaaactgcacctccatcagtggcgatctccacatcctgccggtggcatttaggggtgactccttcacacatactcctcctctggatccacaggaactggatattctgaaaaccgtaaaggaaatcacagggtttttgctgattcaggcttggcctgaaaacaggacggacctccatgcctttgagaacctagaaatcatacgcggcaggaccaagcaacatggtcagttttctcttgcagtcgtcagcctgaacataacatccttgggattacgctccctcaaggagataagtgatggagatgtgataatttcaggaaacaaaaatttgtgctatgcaaatacaataaactggaaaaaactgtttgggacctccggtcagaaaaccaaaattataagcaacagaggtgaaaacagctgcaaggccacaggccaggtctgccatgccttgtgctcccccgagggctgctggggcccggagcccagggactgcgtctcttgccggaatgtcagccgaggcagggaatgcgtggacaagtgcaaccttctggagggtgagccaagggagtttgtggagaactctgagtgcatacagtgccacccagagtgcctgcctcaggccatgaacatcacctgcacaggacggggaccagacaactgtatccagtgtgcccactacattgacggcccccactgcgtcaagacctgcccggcaggagtcatgggagaaaacaacaccctggtctggaagtacgcagacgccggccatgtgtgccacctgtgccatccaaactgcacctacggatgcactgggccaggtcttgaaggctgtccaacgaatgggcctaagatcccgtccatcgccactgggatggtgggggccctcctcttgctgctggtggtggccctggggatcggcctcttcatgcgaaggcgccacatcgttcggaagcgcacgctgcggaggctgctgcaggagagggagcttgtggagcctcttacacccagtggagaagctcccaaccaagctctcttgaggatcttgaaggaaactgaattcaaaaagatcaaagtgctgggctccggtgcgttcggcacggtgtataagggactctggatcccagaaggtgagaaagttaaaattcccgtcgctatcaagacatctccgaaagccaacaaggaaatcctcgatgagcctacgtgatggccagcgtggacaacccccacgtgtgccgcctgctgggcatctgcctcacctccaccgtgcagctcatcacgcagctcatgcccttcggctgcctcctggactatgtccgggaacacaaagacaatattggctcccagtacctgctcaactggtgtgtgcagatcgcaaagggcatgaactacttggaggaccgtcgcttggtgcaccgcgacctggcagccaggaacgtactggtgaaaacaccgcagcatgtcaagatcacagattttgggctggccaaactgctgggtgcggaagagaaagaataccatgcagaaggaggcaaagtgcctatcaagtggatggcattggaatcaattttacacagaatctatacccaccagagtgatgtctggagctacggggtgaccgtttgggagttgatgacctttggatccaagccatatgacggaatccctgccagcgagatctcctccatcctggagaaaggagaacgcctccctcagccacccatatgtaccatcgatgtctacatgatcatggtcaagtgctggatgatagacgcagatagtcgcccaaagttccgtgagttgatcatcgaattctccaaaatggcccgagacccccagcgctaccttgtcattcagggggatgaaagaatgcatttgccaagtcctacagactccaacttctaccgtgccctgatggatgaagaagacatggacgacgtggtggatgccgacgagtacctcatcccacagcagggcttcttcagcagcccctccacgtcacggactcccctcctgagctctctgagtgcaaccagcaacaattccaccgtggcttgcattgatagaaatgggctgcaaagctgtcccatcaaggaagacagcttcttgcagcgatacagctcagaccccacaggcgccttgactgaggacagcatagacgacaccttcctcccagtgcctggtgagtggcttgtctggaaacagtcctgctcctcaacctcctcgacccactcagcagcagccagtctccagtgtccaagccaggtgctccctccagcatctccagagggggaaacagtggcagatttgcagacacagtga

SEQ ID NO: 4 - DNA, 3259 bp, Homo sapiens
atgcgaccctccgggacggccggggcagcgctcctggcgctgctggctgcgctctgcccggcgagtcgggctctggaggaaaagaaagtttgccaaggcacgagtaacaagctcacgcagttgggcacttttgaagatcattttctcagcctccagaggatgttcaataactgtgaggtggtccttgggaatttggaaattacctatgtgcagaggaattatgatctttccttcttaaagaccatccaggaggtggctggttatgtcctcattgccctcaacacagtggagcgaattcctttggaaaacctgcagatcatcagaggaaatatgtactacgaaaattcctatgccttagcagtcttatctaactatgatgcaaataaaaccggactgaaggagctgcccatgagaaatttacagggacaaaagtgtgatccaagctgtcccaatgggagctgctggggtgcaggagaggagaactgccagaaactgaccaaaatcatctgtgcccagcagtgctccgggcgctgccgtggcaagtcccccagtgactgctgccacaaccagtgtgctgcaggctgcacaggcccccgggagagcgactgcctggtctgccgcaaattccgagacgaagccacgtgcaaggacacctgccccccactcatgctctacaaccccaccacgtaccagatggatgtgaaccccgagggcaaatacagctttggtgccacctgcgtgaagaagtgtccccgtaattatgtggtgacagatcacggctcgtgcgtccgagcctgtggggccgacagctatgagatggaggaagacggcgtccgcaagtgtaagaagtgcgaagggccttgccgcaaagtgtgtaacggaataggtattggtgaatttaaagactcactctccataaatgctacgaatattaaacacttcaaaaactgcacctccatcagtggcgatctccacatcctgccggtggcatttaggggtgactccttcacacatactcctcctctggatccacaggaactggatattctgaaaaccgtaaaggaaatcacagggtttttgctgattcaggcttggcctgaaaacaggacggacctccatgcctttgagaacctagaaatcatacgcggcaggaccaagcaacatggtcagttttctcttgcagtcgtcagcctgaacataacatccttgggattacgctccctcaaggagataagtgatggagatgtgataatttcaggaaacaaaaatttgtgctatgcaaatacaataaactggaaaaaactgtttgggacctccggtcagaaaaccaaaattataagcaacagaggtgaaaacagctgcaaggccacaggccaggtctgccatgccttgtgctcccccgagggctgctggggcccggagcccagggactgcgtctcttgccggaatgtcagccgaggcagggaatgcgtggacaagtgcaaccttctggagggtgagccaagggagtttgtggagaactctgagtgcatacagtgccacccagagtgcctgcctcaggccatgaacatcacctgcacaggacggggaccagacaactgtatccagtgtgcccactacattgacggcccccactgcgtcaagacctgcccggcaggagtcatgggagaaaacaacaccctggtctggaagtacgcagacgccggccatgtgtgccacctgtgccatccaaactgcacctacggatgcactgggccaggtcttgaaggctgtccaacgaatgggcctaagatcccgtccatcgccactgggatggtgggggccctcctcttgctgctggtggtggccctggggatcggcctcttcatgcgaaggcgccacatcgttcggaagcgcacgctgcggaggctgctgcaggagagggagcttgtggagcctcttacacccagtggagaagctcccaaccaagctctcttgaggatcttgaaggaaactgaattcaaaaagatcaaagtgctgggctccggtgcgttcggcacggtgtataagggactctggatcccagaaggtgagaaagttaaaattcccgtcgctatcaagcatctccgaaagccaacaaggaaatcctcgatgagcctacgtgatggccagcgtggacaacccccacgtgtgccgcctgctgggcatctgcctcacctccaccgtgcagctcatcacgcagctcatgcccttcggctgcctcctggactatgtccgggaacacaaagacaatattggctcccagtacctgctcaactggtgtgtgcagatcgcaaagggcatgaactacttggaggaccgtcgcttggtgcaccgcgacctggcagccaggaacgtactggtgaaaacaccgcagcatgtcaagatcacagattttgggctggccaaactgctgggtgcggaagagaaagaataccatgcagaaggaggcaaagtgcctatcaagtggatggcattggaatcaattttacacagaatctatacccaccagagtgatgtctggagctacggggtgaccgtttgggagttgatgacctttggatccaagccatatgacggaatccctgccagcgagatctcctccatcctggagaaaggagaacgcctccctcagccacccatatgtaccatcgatgtctacatgatcatggtcaagtgctggatgatagacgcagatagtcgcccaaagttccgtgagttgatcatcgaattctccaaaatggcccgagacccccagcgctaccttgtcattcagggggatgaaagaatgcatttgccaagtcctacagactccaacttctaccgtgccctgatggatgaagaagacatggacgacgtggtggatgccgacgagtacctcatcccacagcagggcttcttcagcagcccctccacgtcacggactcccctcctgagctctctgagtgcaaccagcaacaattccaccgtggcttgcattgatagaaatgggctgcaaagctgtcccatcaaggaagacagcttcttgcagcgatacagctcagaccccacaggcgccttgactgaggacagcatagacgacaccttcctcccagtgcctggtgagtggcttgtctggaaacagtcctgctcctcaacctcctcgacccactcagcagcagccagtctccagtgtccaagccaggtgctccctccagcatctccagagggggaaacagtggcagatttgcagacacagtga

SEQ ID NO: 5 - DNA, 3276 bp, Homo sapiens
atgcgaccctccgggacggccggggcagcgctcctggcgctgctggctgcgctctgcccggcgagtcgggctctggaggaaaagaaagtttgccaaggcacgagtaacaagctcacgcagttgggcacttttgaagatcattttctcagcctccagaggatgttcaataactgtgaggtggtccttgggaatttggaaattacctatgtgcagaggaattatgatctttccttcttaaagaccatccaggaggtggctggttatgtcctcattgccctcaacacagtggagcgaattcctttggaaaacctgcagatcatcagaggaaatatgtactacgaaaattcctatgccttagcagtcttatctaactatgatgcaaataaaaccggactgaaggagctgcccatgagaaatttacagggacaaaagtgtgatccaagctgtcccaatgggagctgctggggtgcaggagaggagaactgccagaaactgaccaaaatcatctgtgcccagcagtgctccgggcgctgccgtggcaagtcccccagtgactgctgccacaaccagtgtgctgcaggctgcacaggcccccgggagagcgactgcctggtctgccgcaaattccgagacgaagccacgtgcaaggacacctgccccccactcatgctctacaaccccaccacgtaccagatggatgtgaaccccgagggcaaatacagctttggtgccacctgcgtgaagaagtgtccccgtaattatgtggtgacagatcacggctcgtgcgtccgagcctgtggggccgacagctatgagatggaggaagacggcgtccgcaagtgtaagaagtgcgaagggccttgccgcaaagtgtgtaacggaataggtattggtgaatttaaagactcactctccataaatgctacgaatattaaacacttcaaaaactgcacctccatcagtggcgatctccacatcctgccggtggcatttaggggtgactccttcacacatactcctcctctggatccacaggaactggatattctgaaaaccgtaaaggaaatcacagggtttttgctgattcaggcttggcctgaaaacaggacggacctccatgcctttgagaacctagaaatcatacgcggcaggaccaagcaacatggtcagttttctcttgcagtcgtcagcctgaacataacatccttgggattacgctccctcaaggagataagtgatggagatgtgataatttcaggaaacaaaaatttgtgctatgcaaatacaataaactggaaaaaactgtttgggacctccggtcagaaaaccaaaattataagcaacagaggtgaaaacagctgcaaggccacaggccaggtctgccatgccttgtgctcccccgagggctgctggggcccggagcccagggactgcgtctcttgccggaatgtcagccgaggcagggaatgcgtggacaagtgcaaccttctggagggtgagccaagggagtttgtggagaactctgagtgcatacagtgccacccagagtgcctgcctcaggccatgaacatcacctgcacaggacggggaccagacaactgtatccagtgtgcccactacattgacggcccccactgcgtcaagacctgcccggcaggagtcatgggagaaaacaacaccctggtctggaagtacgcagacgccggccatgtgtgccacctgtgccatccaaactgcacctacggatgcactgggccaggtcttgaaggctgtccaacgaatgggcctaagatcccgtccatcgccactgggatggtgggggccctcctcttgctgctggtggtggccctggggatcggcctcttcatgcgaaggcgccacatcgttcggaagcgcacgctgcggaggctgctgcaggagagggagcttgtggagcctcttacacccagtggagaagctcccaaccaagctctcttgaggatcttgaaggaaactgaattcaaaaagatcaaagtgctgggctccggtgcgttcggcacggtgtataagggactctggatcccagaaggtgagaaagttaaaattcccgtcgctatcaaggaattaagagaagcaacatctccgaaagccaacaaggaaatcctcgatgaagcctacgtgatggccagcgtggacaacccccacgtgtgccgcctgctgggcatctgcctcacctccaccgtgcagctcatcacgcagctcatgcccttcggctgcctcctggactatgtccgggaacacaaagacaatattggctcccagtacctgctcaactggtgtgtgcagatcgcaaagggcatgaactacttggaggaccgtcgcttggtgcaccgcgacctggcagccaggaacgtactggtgaaaacaccgcagcatgtcaagatcacagattttgggctggccaaactgctgggtgcggaagagaaagaataccatgcagaaggaggcaaagtgcctatcaagtggatggcattggaatcaattttacacagaatctatacccaccagagtgatgtctggagctacggggtgaccgtttgggagttgatgacctttggatccaagccatatgacggaatccctgccagcgagatctcctccatcctggagaaaggagaacgcctccctcagccacccatatgtaccatcgatgtctacatgatcatggtcaagtgctggatgatagacgcagatagtcgcccaaagttccgtgagttgatcatcgaattctccaaaatggcccgagacccccagcgctaccttgtcattcagggggatgaaagaatgcatttgccaagtcctacagactccaacttctaccgtgccctgatggatgaagaagacatggacgacgtggtggatgccgacgagtacctcatcccacagcagggcttcttcagcagcccctccacgtcacggactcccctcctgagctctctgagtgcaaccagcaacaattccaccgtggcttgcattgatagaaatgggctgcaaagctgtcccatcaaggaagacagcttcttgcagcgatacagctcagaccccacaggcgccttgactgaggacagcatagacgacaccttcctcccagtgcctggtgagtggcttgtctggaaacagtcctgctcctcaacctcctcgacccactcagcagcagccagtctccagtgtccaagccaggtgctccctccagcatctccagagggggaaacagtggcagatttgcagacacagtga

SEQ ID NO: 6 - protein, 93 aa, Enterobacteria Phage T4
MGKSGIYQIKNTLNNKVYVGSAKDFEKRWKRHFKDLEKGCHSSIKLQRSFNKHGNVFECSILEEIPYEKDLIIERENFWIKELNSKINGYNIA

SEQ ID NO: 7 - protein, 83 aa, Artificial Sequence
  V117F Mutated Linker
DATFGDTCSTHPLKEEIIKKRSETFKAKMLKLGPDGRKALYSKPGSKNGRWNPETHKFCKCGVRIQTSAYTCSKCRNGGSGGS

SEQ ID NO: 8 - protein, 83 aa, Artificial Sequence
  V117F K135R N140S Mutated Linker
DATFGDTCSTHPLKEEIIKKRSETVKAKMLKLGPDGRKALYSRPGSKSGRWNPETHKFCKCGVRIQTSAYTCSKCRNGGSGGS

SEQ ID NO: 9 - protein, 83 aa, Artificial Sequence
  Linker Domain Variant
DATFGDTCSTHPLKEEIIKKRSETFKAKMLKLGPDGRKALYSRPGSKSGRWNPETHKFCKCGVRIQTSAYTCSKCRNGGSGGS

SEQ ID NO: 10 - protein, 86 aa, Artificial Sequence
  Linker Domain Variant
DATFGDTCSTHPLKEEIIKKRSETVKAKMLKLGPDGRKALYSRPGSKSGRWNPETHKFCKCGVRIQTSAYTCSKCRNGGSGGTGGS

SEQ ID NO: 11 - protein, 87 aa, Artificial Sequence
  Linker Domain Variant
DATFGDTCSTHPLKEEIIKKRSETVKAKMLKLGPDGRKALYSRPGSKSGRWNPETHKFCKCGVRIQTSAYTCSKCRNGGGGSGGGGS

SEQ ID NO: 12 - protein, 95 aa, Artificial Sequence
  Linker Domain Variant
DATFGDTCSTHPLKEEIIKKRSETVKAKMLKLGPDGRKALYSRPGSKSGRWNPETHKFCKCGVRIQTSAYTCSKCRNKESGSVSSEQLAQFRSLD

SEQ ID NO: 13 - protein, 1053 aa, Staphylococcus aureus
MKRNYILGLDIGITSVGYGIIDYETRDVIDAGVRLFKEANVENNEGRRSKRGARRLKRRRRHRIQRVKKLLFDYNLLTDHSELSGINPYEARVKGLSQKLSEEEFSAALLHLAKRRGVHNVNEVEEDTGNELSTKEQISRNSKALEEKYVAELQLERLKKDGEVRGSINRFKTSDYVKEAKQLLKVQKAYHQLDQSFIDTYIDLLETRRTYYEGPGEGSPFGWKDIKEWYEMLMGHCTYFPEELRSVKYAYNADLYNALNDLNNLVITRDENEKLEYYEKFQIIENVFKQKKKPTLKQIAKEILVNEEDIKGYRVTSTGKPEFTNLKVYHDIKDITARKEIIENAELLDQIAKILTIYQSSEDIQEELTNLNSELTQEEIEQISNLKGYTGTHNLSLKAINLILDELWHTNDNQIAIFNRLKLVPKKVDLSQQKEIPTTLVDDFILSPVVKRSFIQSIKVINAIIKKYGLPNDIIIELAREKNSKDAQKMINEMQKRNRQTNERIEEIIRTTGKENAKYLIEKIKLHDMQEGKCLYSLEAIPLEDLLNNPFNYEVDHIIPRSVSFDNSFNNKVLVKQEENSKKGNRTPFQYLSSSDSKISYETFKKHILNLAKGKGRISKTKKEYLLEERDINRFSVQKDFINRNLVDTRYATRGLMNLLRSYFRVNNLDVKVKSINGGFTSFLRRKWKFKKERNKGYKHHAEDALIIANADFIFKEWKKLDKAKKVMENQMFEEKQAESMPEIETEQEYKEIFITPHQIKHIKDFKDYKYSHRVDKKPNRELINDTLYSTRKDDKGNTLIVNNLNGLYDKDNDKLKKLINKSPEKLLMYHHDPQTYQKLKLIMEQYGDEKNPLYKYYEETGNYLTKYSKKDNGPVIKKIKYYGNKLNAHLDITDDYPNSRNKVVKLSLKPYRFDVYLDNGVYKFVTVKNLDVIKKENYYEVNSKCYEEAKKLKKISNQAEFIASFYNNDLIKINGELYRVIGVNNDLLNRIEVNMIDITYREYLENMNDKRPPRIIKTIASKTQSIKKYSTDILGNLYEVKSKKHPQIIKKG

SEQ ID NO: 14 - protein, 1053 aa, Artificial Sequence
  SACAS9 D10E Mutant
MKRNYILGLEIGITSVGYGIIDYETRDVIDAGVRLFKEANVENNEGRRSKRGARRLKRRRRHRIQRVKKLLFDYNLLTDHSELSGINPYEARVKGLSQKLSEEEFSAALLHLAKRRGVHNVNEVEEDTGNELSTKEQISRNSKALEEKYVAELQLERLKKDGEVRGSINRFKTSDYVKEAKQLLKVQKAYHQLDQSFIDTYIDLLETRRTYYEGPGEGSPFGWKDIKEWYEMLMGHCTYFPEELRSVKYAYNADLYNALNDLNNLVITRDENEKLEYYEKFQIIENVFKQKKKPTLKQIAKEILVNEEDIKGYRVTSTGKPEFTNLKVYHDIKDITARKEIIENAELLDQIAKILTIYQSSEDIQEELTNLNSELTQEEIEQISNLKGYTGTHNLSLKAINLILDELWHTNDNQIAIFNRLKLVPKKVDLSQQKEIPTTLVDDFILSPVVKRSFIQSIKVINAIIKKYGLPNDIIIELAREKNSKDAQKMINEMQKRNRQTNERIEEIIRTTGKENAKYLIEKIKLHDMQEGKCLYSLEAIPLEDLLNNPFNYEVDHIIPRSVSFDNSFNNKVLVKQEENSKKGNRTPFQYLSSSDSKISYETFKKHILNLAKGKGRISKTKKEYLLEERDINRFSVQKDFINRNLVDTRYATRGLMNLLRSYFRVNNLDVKVKSINGGFTSFLRRKWKFKKERNKGYKHHAEDALIIANADFIFKEWKKLDKAKKVMENQMFEEKQAESMPEIETEQEYKEIFITPHQIKHIKDFKDYKYSHRVDKKPNRELINDTLYSTRKDDKGNTLIVNNLNGLYDKDNDKLKKLINKSPEKLLMYHHDPQTYQKLKLIMEQYGDEKNPLYKYYEETGNYLTKYSKKDNGPVIKKIKYYGNKLNAHLDITDDYPNSRNKVVKLSLKPYRFDVYLDNGVYKFVTVKNLDVIKKENYYEVNSKCYEEAKKLKKISNQAEFIASFYNNDLIKINGELYRVIGVNNDLLNRIEVNMIDITYREYLENMNDKRPPRIIKTIASKTQSIKKYSTDILGNLYEVKSKKHPQIIKKG

SEQ ID NO: 15 - RNA, 21 nt, Artificial Sequence
  Targets CFTR Gene
gcgucaucaaagcaugccaac

SEQ ID NO: 16 - RNA, 22 nt, Artificial Sequence
  Targets EGFR Gene
aagccaacaaggaaauccucga

SEQ ID NO: 17 - protein, 1053 aa, Artificial Sequence
  SACAS9 D10E + H557A Mutant
MKRNYILGLEIGITSVGYGIIDYETRDVIDAGVRLFKEANVENNEGRRSKRGARRLKRRRRHRIQRVKKLLFDYNLLTDHSELSGINPYEARVKGLSQKLSEEEFSAALLHLAKRRGVHNVNEVEEDTGNELSTKEQISRNSKALEEKYVAELQLERLKKDGEVRGSINRFKTSDYVKEAKQLLKVQKAYHQLDQSFIDTYIDLLETRRTYYEGPGEGSPFGWKDIKEWYEMLMGHCTYFPEELRSVKYAYNADLYNALNDLNNLVITRDENEKLEYYEKFQIIENVFKQKKKPTLKQIAKEILVNEEDIKGYRVTSTGKPEFTNLKVYHDIKDITARKEIIENAELLDQIAKILTIYQSSEDIQEELTNLNSELTQEEIEQISNLKGYTGTHNLSLKAINLILDELWHTNDNQIAIFNRLKLVPKKVDLSQQKEIPTTLVDDFILSPVVKRSFIQSIKVINAIIKKYGLPNDIIIELAREKNSKDAQKMINEMQKRNRQTNERIEEIIRTTGKENAKYLIEKIKLHDMQEGKCLYSLEAIPLEDLLNNPFNYEVDAIIPRSVSFDNSFNNKVLVKQEENSKKGNRTPFQYLSSSDSKISYETFKKHILNLAKGKGRISKTKKEYLLEERDINRFSVQKDFINRNLVDTRYATRGLMNLLRSYFRVNNLDVKVKSINGGFTSFLRRKWKFKKERNKGYKHHAEDALIIANADFIFKEWKKLDKAKKVMENQMFEEKQAESMPEIETEQEYKEIFITPHQIKHIKDFKDYKYSHRVDKKPNRELINDTLYSTRKDDKGNTLIVNNLNGLYDKDNDKLKKLINKSPEKLLMYHHDPQTYQKLKLIMEQYGDEKNPLYKYYEETGNYLTKYSKKDNGPVIKKIKYYGNKLNAHLDITDDYPNSRNKVVKLSLKPYRFDVYLDNGVYKFVTVKNLDVIKKENYYEVNSKCYEEAKKLKKISNQAEFIASFYNNDLIKINGELYRVIGVNNDLLNRIEVNMIDITYREYLENMNDKRPPRIIKTIASKTQSIKKYSTDILGNLYEVKSKKHPQIIKKG

SEQ ID NO: 18 - protein, 1053 aa, Artificial Sequence
  SACAS9 D10A + H557A Mutant
MKRNYILGLAIGITSVGYGIIDYETRDVIDAGVRLFKEANVENNEGRRSKRGARRLKRRRRHRIQRVKKLLFDYNLLTDHSELSGINPYEARVKGLSQKLSEEEFSAALLHLAKRRGVHNVNEVEEDTGNELSTKEQISRNSKALEEKYVAELQLERLKKDGEVRGSINRFKTSDYVKEAKQLLKVQKAYHQLDQSFIDTYIDLLETRRTYYEGPGEGSPFGWKDIKEWYEMLMGHCTYFPEELRSVKYAYNADLYNALNDLNNLVITRDENEKLEYYEKFQIIENVFKQKKKPTLKQIAKEILVNEEDIKGYRVTSTGKPEFTNLKVYHDIKDITARKEIIENAELLDQIAKILTIYQSSEDIQEELTNLNSELTQEEIEQISNLKGYTGTHNLSLKAINLILDELWHTNDNQIAIFNRLKLVPKKVDLSQQKEIPTTLVDDFILSPVVKRSFIQSIKVINAIIKKYGLPNDIIIELAREKNSKDAQKMINEMQKRNRQTNERIEEIIRTTGKENAKYLIEKIKLHDMQEGKCLYSLEAIPLEDLLNNPFNYEVDAIIPRSVSFDNSFNNKVLVKQEENSKKGNRTPFQYLSSSDSKISYETFKKHILNLAKGKGRISKTKKEYLLEERDINRFSVQKDFINRNLVDTRYATRGLMNLLRSYFRVNNLDVKVKSINGGFTSFLRRKWKFKKERNKGYKHHAEDALIIANADFIFKEWKKLDKAKKVMENQMFEEKQAESMPEIETEQEYKEIFITPHQIKHIKDFKDYKYSHRVDKKPNRELINDTLYSTRKDDKGNTLIVNNLNGLYDKDNDKLKKLINKSPEKLLMYHHDPQTYQKLKLIMEQYGDEKNPLYKYYEETGNYLTKYSKKDNGPVIKKIKYYGNKLNAHLDITDDYPNSRNKVVKLSLKPYRFDVYLDNGVYKFVTVKNLDVIKKENYYEVNSKCYEEAKKLKKISNQAEFIASFYNNDLIKINGELYRVIGVNNDLLNRIEVNMIDITYREYLENMNDKRPPRIIKTIASKTQSIKKYSTDILGNLYEVKSKKHPQIIKKG

SEQ ID NO: 19 - protein, 1368 aa, Artificial Sequence
  SPCAS9 D10E, D1135E, R1335Q, T1337R Mutant
MDKKYSIGLEIGTNSVGWAVITDEYKVPSKKFKVLGNTDRHSIKKNLIGALLFDSGETAEATRLKRTARRRYTRRKNRICYLQEIFSNEMAKVDDSFFHRLEESFLVEEDKKHERHPIFGNIVDEVAYHEKYPTIYHLRKKLVDSTDKADLRLIYLALAHMIKFRGHFLIEGDLNPDNSDVDKLFIQLVQTYNQLFEENPINASGVDAKAILSARLSKSRRLENLIAQLPGEKKNGLFGNLIALSLGLTPNFKSNFDLAEDAKLQLSKDTYDDDLDNLLAQIGDQYADLFLAAKNLSDAILLSDILRVNTEITKAPLSASMIKRYDEHHQDLTLLKALVRQQLPEKYKEIFFDQSKNGYAGYIDGGASQEEFYKFIKPILEKMDGTEELLVKLNREDLLRKQRTFDNGSIPHQIHLGELHAILRRQEDFYPFLKDNREKIEKILTFRIPYYVGPLARGNSRFAWMTRKSEETITPWNFEEVVDKGASAQSFIERMTNFDKNLPNEKVLPKHSLLYEYFTVYNELTKVKYVTEGMRKPAFLSGEQKKAIVDLLFKTNRKVTVKQLKEDYFKKIECFDSVEISGVEDRFNASLGTYHDLLKIIKDKDFLDNEENEDILEDIVLTLTLFEDREMIEERLKTYAHLFDDKVMKQLKRRRYTGWGRLSRKLINGIRDKQSGKTILDFLKSDGFANRNFMQLIHDDSLTFKEDIQKAQVSGQGDSLHEHIANLAGSPAIKKGILQTVKVVDELVKVMGRHKPENIVIEMARENQTTQKGQKNSRERMKRIEEGIKELGSQILKEHPVENTQLQNEKLYLYYLQNGRDMYVDQELDINRLSDYDVDHIVPQSFLKDDSIDNKVLTRSDKNRGKSDNVPSEEVVKKMKNYWRQLLNAKLITQRKFDNLTKAERGGLSELDKAGFIKRQLVETRQITKHVAQILDSRMNTKYDENDKLIREVKVITLKSKLVSDFRKDFQFYKVREINNYHHAHDAYLNAVVGTALIKKYPKLESEFVYGDYKVYDVRKMIAKSEQEIGKATAKYFFYSNIMNFFKTEITLANGEIRKRPLIETNGETGEIVWDKGRDFATVRKVLSMPQVNIVKKTEVQTGGFSKESILPKRNSDKLIARKKDWDPKKYGGFESPTVAYSVLVVAKVEKGKSKKLKSVKELLGITIMERSSFEKNPIDFLEAKGYKEVKKDLIIKLPKYSLFELENGRKRMLASAGELQKGNELALPSKYVNFLYLASHYEKLKGSPEDNEQKQLFVEQHKHYLDEIIEQISEFSKRVILADANLDKVLSAYNKHRDKPIREQAENIIHLFTLTNLGAPAAFKYFDTTIDRKQYRSTKEVLDATLIHQSITGLYETRIDLSQLGGD

SEQ ID NO: 20 - protein, 1368 aa, Artificial Sequence
  SPCAS9 D10E, H840A, D1135E, R1335Q, T1337R Mutant
MDKKYSIGLEIGTNSVGWAVITDEYKVPSKKFKVLGNTDRHSIKKNLIGALLFDSGETAEATRLKRTARRRYTRRKNRICYLQEIFSNEMAKVDDSFFHRLEESFLVEEDKKHERHPIFGNIVDEVAYHEKYPTIYHLRKKLVDSTDKADLRLIYLALAHMIKFRGHFLIEGDLNPDNSDVDKLFIQLVQTYNQLFEENPINASGVDAKAILSARLSKSRRLENLIAQLPGEKKNGLFGNLIALSLGLTPNFKSNFDLAEDAKLQLSKDTYDDDLDNLLAQIGDQYADLFLAAKNLSDAILLSDILRVNTEITKAPLSASMIKRYDEHHQDLTLLKALVRQQLPEKYKEIFFDQSKNGYAGYIDGGASQEEFYKFIKPILEKMDGTEELLVKLNREDLLRKQRTFDNGSIPHQIHLGELHAILRRQEDFYPFLKDNREKIEKILTFRIPYYVGPLARGNSRFAWMTRKSEETITPWNFEEVVDKGASAQSFIERMTNFDKNLPNEKVLPKHSLLYEYFTVYNELTKVKYVTEGMRKPAFLSGEQKKAIVDLLFKTNRKVTVKQLKEDYFKKIECFDSVEISGVEDRFNASLGTYHDLLKIIKDKDFLDNEENEDILEDIVLTLTLFEDREMIEERLKTYAHLFDDKVMKQLKRRRYTGWGRLSRKLINGIRDKQSGKTILDFLKSDGFANRNFMQLIHDDSLTFKEDIQKAQVSGQGDSLHEHIANLAGSPAIKKGILQTVKVVDELVKVMGRHKPENIVIEMARENQTTQKGQKNSRERMKRIEEGIKELGSQILKEHPVENTQLQNEKLYLYYLQNGRDMYVDQELDINRLSDYDVDAIVPQSFLKDDSIDNKVLTRSDKNRGKSDNVPSEEVVKKMKNYWRQLLNAKLITQRKFDNLTKAERGGLSELDKAGFIKRQLVETRQITKHVAQILDSRMNTKYDENDKLIREVKVITLKSKLVSDFRKDFQFYKVREINNYHHAHDAYLNAVVGTALIKKYPKLESEFVYGDYKVYDVRKMIAKSEQEIGKATAKYFFYSNIMNFFKTEITLANGEIRKRPLIETNGETGEIVWDKGRDFATVRKVLSMPQVNIVKKTEVQTGGFSKESILPKRNSDKLIARKKDWDPKKYGGFESPTVAYSVLVVAKVEKGKSKKLKSVKELLGITIMERSSFEKNPIDFLEAKGYKEVKKDLIIKLPKYSLFELENGRKRMLASAGELQKGNELALPSKYVNFLYLASHYEKLKGSPEDNEQKQLFVEQHKHYLDEIIEQISEFSKRVILADANLDKVLSAYNKHRDKPIREQAENIIHLFTLTNLGAPAAFKYFDTTIDRKQYRSTKEVLDATLIHQSITGLYETRIDLSQLGGD